European Patent Application EP 4 123 025 A1, published January 25, 2023. Title: Variant of thermostable mismatch endonuclease. Applicant: TAKARA BIO INC. EDUCATIONAL CORPORATION KANSAI BUNRI SOUGOUGAKUEN KYUSHU UNIVERSITY, NATIONAL UNIVERSITY CORPORATION. The sequence listing filed with the application follows.

SEQUENCE LISTING (36 sequences)

SEQ ID NO: 1 - protein, 267 aa, Pyrococcus furiosus
MEMTKAIVKENPRIEEIKELLEVAESREGLLTIFARCTVYYEGRAKSELGEGDRIIIIKPDGSFLIHQKKKREPVNWQPPGSKVKMEGNSLISIRRNPKETLKVDIIEAYAAVLFMAEDYEELTLTGSEAEMAELIFQNPNVIEEGFKPMFREKPIKHGIVDVLGVDREGNIVVLELKRRRADLHAVSQLKRYVDALKEEHGNKVRGILVAPSLTEGAKKLLEKLGLEFRKLEPPKKGKKKSSKQKTLDFLNDTVRITGASPPEAIQ

SEQ ID NO: 2 - protein, 267 aa, Artificial Sequence
  Amino acid sequence of mismatch endonuclease PF0012 W77F variant
MEMTKAIVKENPRIEEIKELLEVAESREGLLTIFARCTVYYEGRAKSELGEGDRIIIIKPDGSFLIHQKKKREPVNFQPPGSKVKMEGNSLISIRRNPKETLKVDIIEAYAAVLFMAEDYEELTLTGSEAEMAELIFQNPNVIEEGFKPMFREKPIKHGIVDVLGVDREGNIVVLELKRRRADLHAVSQLKRYVDALKEEHGNKVRGILVAPSLTEGAKKLLEKLGLEFRKLEPPKKGKKKSSKQKTLDFLNDTVRITGASPPEAIQ

SEQ ID NO: 3 - protein, 251 aa, Thermococcus barophilus
MEAKVEPSHEEIIEILDKALSVEAIITLFAYCRVFYEGRAKSELGPGDRVIIIKPDGSFLIHQKNKREPVNWQPPGSVVSIVLEDGRIMLRSVRRKPKETLEVELIKTYLVSYFQAEDYEELTLTGSEAEMADLIFENPSLIEEGFKPLFKEKPIKHGIVDVLGKDKHGNLVVLELKRRRADLHAVSQLKRYVDSLREEHKNVRGILVAPSLTAGAKKLLEKEGLEFKKLNPPKREKRKKGKQKTLDFLSP

SEQ ID NO: 4 - protein, 263 aa, Methanocaldococcus jannaschii
MMRLEKVFYLTNPTTKDLENFIDMYVFKYILILLARCKVFYEGRAKSQLEEGDRVIIIKPDGAFLIHKDKKREPVNWQPSGSSIIWEVEDNFFILKSIRRKPKEELKVVISEVYHACAFNCEDYEEINLRGSESEMAEMIFRNPDLIEEGFKPISREYQIPTGIVDILGKDKENKWVILELKRRRADLQAVSQLKRYVEYFKNKYGEDKVRGILVSPSLTTGAEKLLKEENLEFKRLNPPKGSKRDLKHNIKTKKTTVLDEWL

SEQ ID NO: 5 - protein, 252 aa, Thermococcus kodakarensis
MSKDKVTVITSPSTEELVSLVNSALLEEAMLTIFARCKVHYDGRAKSELGSGDRVIIVKPDGSFLIHQSKKREPVNWQPPGSRVRLELRENPVLVSIRRKPRETLEVELEEVYMVSVFRAEDYEELALTGSEAEMAELIFENPEVIEPGFKPLFREKAIGTGIVDVLGRDSDGNIVVLELKRRRAELHAVRQLKSYVEILREEYGDKVRGILVAPSLTSGAKRLLEKEGLEFRKLEPPKRDSKKKGRQKTLF

SEQ ID NO: 6 - protein, 267 aa, Artificial Sequence
  Amino acid sequence of mismatch endonuclease variant S47K+N76D from PF0012
MEMTKAIVKENPRIEEIKELLEVAESREGLLTIFARCTVYYEGRAKKELGEGDRIIIIKPDGSFLIHQKKKREPVDWQPPGSKVKMEGNSLISIRRNPKETLKVDIIEAYAAVLFMAEDYEELTLTGSEAEMAELIFQNPNVIEEGFKPMFREKPIKHGIVDVLGVDREGNIVVLELKRRRADLHAVSQLKRYVDALKEEHGNKVRGILVAPSLTEGAKKLLEKLGLEFRKLEPPKKGKKKSSKQKTLDFLNDTVRITGASPPEAIQ

SEQ ID NO: 7 - protein, 267 aa, Artificial Sequence
  Amino acid sequence of mismatch endonuclease variant S47R+N76D+L123A from PF0012
MEMTKAIVKENPRIEEIKELLEVAESREGLLTIFARCTVYYEGRAKRELGEGDRIIIIKPDGSFLIHQKKKREPVDWQPPGSKVKMEGNSLISIRRNPKETLKVDIIEAYAAVLFMAEDYEEATLTGSEAEMAELIFQNPNVIEEGFKPMFREKPIKHGIVDVLGVDREGNIVVLELKRRRADLHAVSQLKRYVDALKEEHGNKVRGILVAPSLTEGAKKLLEKLGLEFRKLEPPKKGKKKSSKQKTLDFLNDTVRITGASPPEAIQ

SEQ ID NO: 8 - protein, 267 aa, Artificial Sequence
  Amino acid sequence of mismatch endonuclease variant S47R+N76D+L123G from PF0012
MEMTKAIVKENPRIEEIKELLEVAESREGLLTIFARCTVYYEGRAKRELGEGDRIIIIKPDGSFLIHQKKKREPVDWQPPGSKVKMEGNSLISIRRNPKETLKVDIIEAYAAVLFMAEDYEEGTLTGSEAEMAELIFQNPNVIEEGFKPMFREKPIKHGIVDVLGVDREGNIVVLELKRRRADLHAVSQLKRYVDALKEEHGNKVRGILVAPSLTEGAKKLLEKLGLEFRKLEPPKKGKKKSSKQKTLDFLNDTVRITGASPPEAIQ

SEQ ID NO: 9 - protein, 267 aa, Artificial Sequence
  Amino acid sequence of mismatch endonuclease variant Q78R+L123S from PF0012
MEMTKAIVKENPRIEEIKELLEVAESREGLLTIFARCTVYYEGRAKSELGEGDRIIIIKPDGSFLIHQKKKREPVNWRPPGSKVKMEGNSLISIRRNPKETLKVDIIEAYAAVLFMAEDYEESTLTGSEAEMAELIFQNPNVIEEGFKPMFREKPIKHGIVDVLGVDREGNIVVLELKRRRADLHAVSQLKRYVDALKEEHGNKVRGILVAPSLTEGAKKLLEKLGLEFRKLEPPKKGKKKSSKQKTLDFLNDTVRITGASPPEAIQ

SEQ ID NO: 10 - protein, 267 aa, Artificial Sequence
  Amino acid sequence of mismatch endonuclease variant Q78R+L123T from PF0012
MEMTKAIVKENPRIEEIKELLEVAESREGLLTIFARCTVYYEGRAKSELGEGDRIIIIKPDGSFLIHQKKKREPVNWRPPGSKVKMEGNSLISIRRNPKETLKVDIIEAYAAVLFMAEDYEETTLTGSEAEMAELIFQNPNVIEEGFKPMFREKPIKHGIVDVLGVDREGNIVVLELKRRRADLHAVSQLKRYVDALKEEHGNKVRGILVAPSLTEGAKKLLEKLGLEFRKLEPPKKGKKKSSKQKTLDFLNDTVRITGASPPEAIQ

SEQ ID NO: 11 - protein, 267 aa, Artificial Sequence
  Amino acid sequence of mismatch endonuclease variant Q78R+L123M from PF0012
MEMTKAIVKENPRIEEIKELLEVAESREGLLTIFARCTVYYEGRAKSELGEGDRIIIIKPDGSFLIHQKKKREPVNWRPPGSKVKMEGNSLISIRRNPKETLKVDIIEAYAAVLFMAEDYEEMTLTGSEAEMAELIFQNPNVIEEGFKPMFREKPIKHGIVDVLGVDREGNIVVLELKRRRADLHAVSQLKRYVDALKEEHGNKVRGILVAPSLTEGAKKLLEKLGLEFRKLEPPKKGKKKSSKQKTLDFLNDTVRITGASPPEAIQ

SEQ ID NO: 12 - protein, 267 aa, Artificial Sequence
  Amino acid sequence of mismatch endonuclease variant Q78R+L123C from PF0012
MEMTKAIVKENPRIEEIKELLEVAESREGLLTIFARCTVYYEGRAKSELGEGDRIIIIKPDGSFLIHQKKKREPVNWRPPGSKVKMEGNSLISIRRNPKETLKVDIIEAYAAVLFMAEDYEECTLTGSEAEMAELIFQNPNVIEEGFKPMFREKPIKHGIVDVLGVDREGNIVVLELKRRRADLHAVSQLKRYVDALKEEHGNKVRGILVAPSLTEGAKKLLEKLGLEFRKLEPPKKGKKKSSKQKTLDFLNDTVRITGASPPEAIQ

SEQ ID NO: 13 - protein, 267 aa, Artificial Sequence
  Amino acid sequence of mismatch endonuclease variant Q78R+L125V from PF0012
MEMTKAIVKENPRIEEIKELLEVAESREGLLTIFARCTVYYEGRAKSELGEGDRIIIIKPDGSFLIHQKKKREPVNWRPPGSKVKMEGNSLISIRRNPKETLKVDIIEAYAAVLFMAEDYEELTVTGSEAEMAELIFQNPNVIEEGFKPMFREKPIKHGIVDVLGVDREGNIVVLELKRRRADLHAVSQLKRYVDALKEEHGNKVRGILVAPSLTEGAKKLLEKLGLEFRKLEPPKKGKKKSSKQKTLDFLNDTVRITGASPPEAIQ

SEQ ID NO: 14 - protein, 267 aa, Artificial Sequence
  Amino acid sequence of mismatch endonuclease variant Q78R+L125A from PF0012
MEMTKAIVKENPRIEEIKELLEVAESREGLLTIFARCTVYYEGRAKSELGEGDRIIIIKPDGSFLIHQKKKREPVNWRPPGSKVKMEGNSLISIRRNPKETLKVDIIEAYAAVLFMAEDYEELTATGSEAEMAELIFQNPNVIEEGFKPMFREKPIKHGIVDVLGVDREGNIVVLELKRRRADLHAVSQLKRYVDALKEEHGNKVRGILVAPSLTEGAKKLLEKLGLEFRKLEPPKKGKKKSSKQKTLDFLNDTVRITGASPPEAIQ

SEQ ID NO: 15 - protein, 542 aa, Artificial Sequence
  Amino acid sequence of mismatch endonuclease variant hetero dimer from variant S47R+N76D+L123A and variant Q78R+L123M
MEMTKAIVKENPRIEEIKELLEVAESREGLLTIFARCTVYYEGRAKRELGEGDRIIIIKPDGSFLIHQKKKREPVDWQPPGSKVKMEGNSLISIRRNPKETLKVDIIEAYAAVLFMAEDYEEATLTGSEAEMAELIFQNPNVIEEGFKPMFREKPIKHGIVDVLGVDREGNIVVLELKRRRADLHAVSQLKRYVDALKEEHGNKVRGILVAPSLTEGAKKLLEKLGLEFRKLEPPKKGKKKSSKQKTLDFLNDTVRITGASPPEAIQLEVLFQGPMEMTKAIVKENPRIEEIKELLEVAESREGLLTIFARCTVYYEGRAKSELGEGDRIIIIKPDGSFLIHQKKKREPVNWRPPGSKVKMEGNSLISIRRNPKETLKVDIIEAYAAVLFMAEDYEEMTLTGSEAEMAELIFQNPNVIEEGFKPMFREKPIKHGIVDVLGVDREGNIVVLELKRRRADLHAVSQLKRYVDALKEEHGNKVRGILVAPSLTEGAKKLLEKLGLEFRKLEPPKKGKKKSSKQKTLDFLNDTVRITGASPPEAIQ

SEQ ID NO: 16 - DNA, 804 bp, Pyrococcus furiosus
atggaaatgaccaaagcgattgtgaaagaaaacccgcgcattgaagaaattaaagaactgctggaagtggcggaaagccgcgaaggcctgctgaccatttttgcgcgctgcaccgtgtattatgaaggccgcgcgaaaagcgaactgggcgaaggcgatcgcattattattattaaaccggatggcagctttctgattcatcagaaaaagaaacgcgaaccggtgaactggcagccgccgggcagcaaagtgaaaatggaaggcaacagcctgattagcattcgccgcaacccgaaagaaaccctgaaagtggatattattgaagcgtatgcggcggtgctgtttatggcggaagattatgaagaactgaccctgaccggcagcgaagcggaaatggcggaactgatttttcagaacccgaacgtgattgaagaaggctttaaaccgatgtttcgcgaaaaaccgattaaacatggcattgtggatgtgctgggcgtggatcgcgaaggcaacattgtggtgctggaactgaaacgccgccgcgcggatctgcatgcggtgagccagctgaaacgctatgtggatgcgctgaaagaagaacatggcaacaaagtgcgcggcattctggtggcgccgagcctgaccgaaggcgcgaaaaaactgctggaaaaactgggcctggaatttcgcaaactggaaccgccgaaaaaaggcaaaaagaaaagcagcaaacagaaaaccctggattttctgaacgataccgtgcgcattaccggcgcgagcccgccggaagcgattcagtaa

SEQ ID NO: 17 - DNA, 804 bp, Artificial Sequence
  Nucleic acid sequence encoding gene of mismatch endonuclease PF0012 W77F variant
atggaaatgaccaaagcgattgtgaaagaaaacccgcgcattgaagaaattaaagaactgctggaagtggcggaaagccgcgaaggcctgctgaccatttttgcgcgctgcaccgtgtattatgaaggccgcgcgaaaagcgaactgggcgaaggcgatcgcattattattattaaaccggatggcagctttctgattcatcagaaaaagaaacgcgaaccggtgaactttcagccgccgggcagcaaagtgaaaatggaaggcaacagcctgattagcattcgccgcaacccgaaagaaaccctgaaagtggatattattgaagcgtatgcggcggtgctgtttatggcggaagattatgaagaactgaccctgaccggcagcgaagcggaaatggcggaactgatttttcagaacccgaacgtgattgaagaaggctttaaaccgatgtttcgcgaaaaaccgattaaacatggcattgtggatgtgctgggcgtggatcgcgaaggcaacattgtggtgctggaactgaaacgccgccgcgcggatctgcatgcggtgagccagctgaaacgctatgtggatgcgctgaaagaagaacatggcaacaaagtgcgcggcattctggtggcgccgagcctgaccgaaggcgcgaaaaaactgctggaaaaactgggcctggaatttcgcaaactggaaccgccgaaaaaaggcaaaaagaaaagcagcaaacagaaaaccctggattttctgaacgataccgtgcgcattaccggcgcgagcccgccggaagcgattcagtaa

SEQ ID NO: 18 - DNA, 756 bp, Thermococcus barophilus
atggaagctaaggttgaaccctctcacgaagaaataattgaaattttggataaagccctctctgttgaggctatcataactctttttgcttattgtagggtattctatgaggggagagccaagagtgagcttggccccggagatagggtcattataatcaagccagatggctcttttttaattcaccagaagaacaaaagagaacctgttaactggcagccgccggggagtgttgtcagcatcgttcttgaggatgggagaataatgctgagaagtgttaggagaaaaccgaaagaaacccttgaagttgagctcattaaaacttatcttgtgagttatttccaagcagaggattatgaggagctgacattaactggaagtgaagcagagatggctgatttgatctttgagaatccctcattaattgaggaaggatttaaaccgctctttaaggaaaagccaattaaacatggaatagttgatgtgcttggaaaagacaaacatggcaatttggttgtccttgagcttaagcgcaggagagcagatctgcatgcggtcagtcaacttaaaagatatgttgattctctgagggaggagcataaaaatgttcgtgggattttggttgccccttctcttacggctggggctaaaaaattacttgaaaaagaagggctggaatttaaaaagctgaatccaccaaagcgtgaaaagaggaaaaaaggcaagcagaaaacccttgattttctcagcccatag

SEQ ID NO: 19 - DNA, 792 bp, Methanocaldococcus jannaschii
atgatgagattggagaaagttttctatctaaccaatcctactaccaaagatttagaaaattttattgatatgtatgtgtttaaatatatattaatattattagctcgatgtaaagttttttatgaaggcagagctaaaagtcagttagaagagggagatagagtcattataataaaaccagatggagcctttttaattcataaagataaaaaaagagaacctgtaaattggcaaccttctggaagtagtataatatgggaagttgaagataactttttcattttaaaaagcattagaagaaagccaaaagaagagttaaaggttgttatttcagaagtttatcatgcatgtgcttttaactgtgaagattatgaagagataaatctaaggggtagtgaatcagagatggcagagatgatttttagaaatccagatttgattgaagaaggatttaagcccatatcaagagagtatcagattcccactggaatcgttgatattttaggaaaagataaagagaataaatgggttatcttagagctaaagagaaggagagctgatttacaggcagtttctcaactaaaaaggtatgtggaatattttaaaaacaaatatggtgaggataaagttagaggaattttggtttctccctctttaactactggggcggaaaaattgctgaaagaggagaacttagaatttaaaagacttaatccaccaaaaggaagtaaaagagatttaaaacataacataaaaactaaaaaaacaacagttttagatgaatggctataa

SEQ ID NO: 20 - DNA, 759 bp, Thermococcus kodakarensis
atgtccaaggataaggtaacggtcatcacgtcgccatcaaccgaagaactcgtttcgctagtcaattcagctctcttagaagaggccatgctgacgatttttgcccgctgtaaggtccactacgatggaagggcaaagagcgagctcggctccggcgatagggtcatcatagtcaagcccgacggctcttttctcatccaccagagcaagaagcgcgagcccgtgaactggcagccaccgggtagcagagtgaggctggagctgagggagaacccagttctcgtctcgataaggagaaagccgagggagacccttgaggtcgagctcgaagaggtctacatggtctccgtcttccgagctgaggactacgaggagctcgcccttacggggagcgaggccgagatggcggagcttatctttgaaaatccagaggtcatagagcctggcttcaagccgctgttcagggagaaggcgataggaactggaatcgttgatgtccttggaagggacagtgatgggaatatagttgtccttgagcttaagcgcaggagggcggaactccatgccgttagacagctcaagagctacgtcgagattctgagagaggagtacggcgataaagtccgtggaattctcgttgctccctcgctcacttctggggcaaaaagactcctggaaaaggagggcctcgagttcaggaagctcgaaccgcctaaaagagactccaaaaagaagggcagacagaagacactgttttag

SEQ ID NO: 21 - DNA, 804 bp, Artificial Sequence
  Nucleic acid sequence encoding gene of mismatch endonuclease variant S47K+N76D from PF0012
atggaaatgaccaaagcgattgtgaaagaaaacccgcgcattgaagaaattaaagaactgctggaagtggcggaaagccgcgaaggcctgctgaccatttttgcgcgctgcaccgtgtattatgaaggccgcgcgaaaaaagaactgggcgaaggcgatcgcattattattattaaaccggatggcagctttctgattcatcagaaaaagaaacgcgaaccggtggattggcagccgccgggcagcaaagtgaaaatggaaggcaacagcctgattagcattcgccgcaacccgaaagaaaccctgaaagtggatattattgaagcgtatgcggcggtgctgtttatggcggaagattatgaagaactgaccctgaccggcagcgaagcggaaatggcggaactgatttttcagaacccgaacgtgattgaagaaggctttaaaccgatgtttcgcgaaaaaccgattaaacatggcattgtggatgtgctgggcgtggatcgcgaaggcaacattgtggtgctggaactgaaacgccgccgcgcggatctgcatgcggtgagccagctgaaacgctatgtggatgcgctgaaagaagaacatggcaacaaagtgcgcggcattctggtggcgccgagcctgaccgaaggcgcgaaaaaactgctggaaaaactgggcctggaatttcgcaaactggaaccgccgaaaaaaggcaaaaagaaaagcagcaaacagaaaaccctggattttctgaacgataccgtgcgcattaccggcgcgagcccgccggaagcgattcagtaa

SEQ ID NO: 22 - DNA, 804 bp, Artificial Sequence
  Nucleic acid sequence encoding gene of mismatch endonuclease variant S47R+N76D+L123A from PF0012
atggaaatgaccaaagcgattgtgaaagaaaacccgcgcattgaagaaattaaagaactgctggaagtggcggaaagccgcgaaggcctgctgaccatttttgcgcgctgcaccgtgtattatgaaggccgcgcgaaacgcgaactgggcgaaggcgatcgcattattattattaaaccggatggcagctttctgattcatcagaaaaagaaacgcgaaccggtggattggcagccgccgggcagcaaagtgaaaatggaaggcaacagcctgattagcattcgccgcaacccgaaagaaaccctgaaagtggatattattgaagcgtatgcggcggtgctgtttatggcggaagattatgaagaagcgaccctgaccggcagcgaagcggaaatggcggaactgatttttcagaacccgaacgtgattgaagaaggctttaaaccgatgtttcgcgaaaaaccgattaaacatggcattgtggatgtgctgggcgtggatcgcgaaggcaacattgtggtgctggaactgaaacgccgccgcgcggatctgcatgcggtgagccagctgaaacgctatgtggatgcgctgaaagaagaacatggcaacaaagtgcgcggcattctggtggcgccgagcctgaccgaaggcgcgaaaaaactgctggaaaaactgggcctggaatttcgcaaactggaaccgccgaaaaaaggcaaaaagaaaagcagcaaacagaaaaccctggattttctgaacgataccgtgcgcattaccggcgcgagcccgccggaagcgattcagtaa

SEQ ID NO: 23 - DNA, 804 bp, Artificial Sequence
  Nucleic acid sequence encoding gene of mismatch endonuclease variant S47R+N76D+L123G from PF0012
atggaaatgaccaaagcgattgtgaaagaaaacccgcgcattgaagaaattaaagaactgctggaagtggcggaaagccgcgaaggcctgctgaccatttttgcgcgctgcaccgtgtattatgaaggccgcgcgaaacgcgaactgggcgaaggcgatcgcattattattattaaaccggatggcagctttctgattcatcagaaaaagaaacgcgaaccggtggattggcagccgccgggcagcaaagtgaaaatggaaggcaacagcctgattagcattcgccgcaacccgaaagaaaccctgaaagtggatattattgaagcgtatgcggcggtgctgtttatggcggaagattatgaagaaggcaccctgaccggcagcgaagcggaaatggcggaactgatttttcagaacccgaacgtgattgaagaaggctttaaaccgatgtttcgcgaaaaaccgattaaacatggcattgtggatgtgctgggcgtggatcgcgaaggcaacattgtggtgctggaactgaaacgccgccgcgcggatctgcatgcggtgagccagctgaaacgctatgtggatgcgctgaaagaagaacatggcaacaaagtgcgcggcattctggtggcgccgagcctgaccgaaggcgcgaaaaaactgctggaaaaactgggcctggaatttcgcaaactggaaccgccgaaaaaaggcaaaaagaaaagcagcaaacagaaaaccctggattttctgaacgataccgtgcgcattaccggcgcgagcccgccggaagcgattcagtaa

SEQ ID NO: 24 - DNA, 804 bp, Artificial Sequence
  Nucleic acid sequence encoding gene of mismatch endonuclease variant Q78R+L123S from PF0012
atggaaatgaccaaagcgattgtgaaagaaaacccgcgcattgaagaaattaaagaactgctggaagtggcggaaagccgcgaaggcctgctgaccatttttgcgcgctgcaccgtgtattatgaaggccgcgcgaaaagcgaactgggcgaaggcgatcgcattattattattaaaccggatggcagctttctgattcatcagaaaaagaaacgcgaaccggtgaactggcgcccgccgggcagcaaagtgaaaatggaaggcaacagcctgattagcattcgccgcaacccgaaagaaaccctgaaagtggatattattgaagcgtatgcggcggtgctgtttatggcggaagattatgaagaaagcaccctgaccggcagcgaagcggaaatggcggaactgatttttcagaacccgaacgtgattgaagaaggctttaaaccgatgtttcgcgaaaaaccgattaaacatggcattgtggatgtgctgggcgtggatcgcgaaggcaacattgtggtgctggaactgaaacgccgccgcgcggatctgcatgcggtgagccagctgaaacgctatgtggatgcgctgaaagaagaacatggcaacaaagtgcgcggcattctggtggcgccgagcctgaccgaaggcgcgaaaaaactgctggaaaaactgggcctggaatttcgcaaactggaaccgccgaaaaaaggcaaaaagaaaagcagcaaacagaaaaccctggattttctgaacgataccgtgcgcattaccggcgcgagcccgccggaagcgattcagtaa

SEQ ID NO: 25 - DNA, 804 bp, Artificial Sequence
  Nucleic acid sequence encoding gene of mismatch endonuclease variant Q78R+L123T from PF0012
atggaaatgaccaaagcgattgtgaaagaaaacccgcgcattgaagaaattaaagaactgctggaagtggcggaaagccgcgaaggcctgctgaccatttttgcgcgctgcaccgtgtattatgaaggccgcgcgaaaagcgaactgggcgaaggcgatcgcattattattattaaaccggatggcagctttctgattcatcagaaaaagaaacgcgaaccggtgaactggcgcccgccgggcagcaaagtgaaaatggaaggcaacagcctgattagcattcgccgcaacccgaaagaaaccctgaaagtggatattattgaagcgtatgcggcggtgctgtttatggcggaagattatgaagaaaccaccctgaccggcagcgaagcggaaatggcggaactgatttttcagaacccgaacgtgattgaagaaggctttaaaccgatgtttcgcgaaaaaccgattaaacatggcattgtggatgtgctgggcgtggatcgcgaaggcaacattgtggtgctggaactgaaacgccgccgcgcggatctgcatgcggtgagccagctgaaacgctatgtggatgcgctgaaagaagaacatggcaacaaagtgcgcggcattctggtggcgccgagcctgaccgaaggcgcgaaaaaactgctggaaaaactgggcctggaatttcgcaaactggaaccgccgaaaaaaggcaaaaagaaaagcagcaaacagaaaaccctggattttctgaacgataccgtgcgcattaccggcgcgagcccgccggaagcgattcagtaa

SEQ ID NO: 26 - DNA, 804 bp, Artificial Sequence
  Nucleic acid sequence encoding gene of mismatch endonuclease variant Q78R+L123M from PF0012
atggaaatgaccaaagcgattgtgaaagaaaacccgcgcattgaagaaattaaagaactgctggaagtggcggaaagccgcgaaggcctgctgaccatttttgcgcgctgcaccgtgtattatgaaggccgcgcgaaaagcgaactgggcgaaggcgatcgcattattattattaaaccggatggcagctttctgattcatcagaaaaagaaacgcgaaccggtgaactggcgcccgccgggcagcaaagtgaaaatggaaggcaacagcctgattagcattcgccgcaacccgaaagaaaccctgaaagtggatattattgaagcgtatgcggcggtgctgtttatggcggaagattatgaagaaatgaccctgaccggcagcgaagcggaaatggcggaactgatttttcagaacccgaacgtgattgaagaaggctttaaaccgatgtttcgcgaaaaaccgattaaacatggcattgtggatgtgctgggcgtggatcgcgaaggcaacattgtggtgctggaactgaaacgccgccgcgcggatctgcatgcggtgagccagctgaaacgctatgtggatgcgctgaaagaagaacatggcaacaaagtgcgcggcattctggtggcgccgagcctgaccgaaggcgcgaaaaaactgctggaaaaactgggcctggaatttcgcaaactggaaccgccgaaaaaaggcaaaaagaaaagcagcaaacagaaaaccctggattttctgaacgataccgtgcgcattaccggcgcgagcccgccggaagcgattcagtaa

SEQ ID NO: 27 - DNA, 804 bp, Artificial Sequence
  Nucleic acid sequence encoding gene of mismatch endonuclease variant Q78R+L123C from PF0012
atggaaatgaccaaagcgattgtgaaagaaaacccgcgcattgaagaaattaaagaactgctggaagtggcggaaagccgcgaaggcctgctgaccatttttgcgcgctgcaccgtgtattatgaaggccgcgcgaaaagcgaactgggcgaaggcgatcgcattattattattaaaccggatggcagctttctgattcatcagaaaaagaaacgcgaaccggtgaactggcgcccgccgggcagcaaagtgaaaatggaaggcaacagcctgattagcattcgccgcaacccgaaagaaaccctgaaagtggatattattgaagcgtatgcggcggtgctgtttatggcggaagattatgaagaatgcaccctgaccggcagcgaagcggaaatggcggaactgatttttcagaacccgaacgtgattgaagaaggctttaaaccgatgtttcgcgaaaaaccgattaaacatggcattgtggatgtgctgggcgtggatcgcgaaggcaacattgtggtgctggaactgaaacgccgccgcgcggatctgcatgcggtgagccagctgaaacgctatgtggatgcgctgaaagaagaacatggcaacaaagtgcgcggcattctggtggcgccgagcctgaccgaaggcgcgaaaaaactgctggaaaaactgggcctggaatttcgcaaactggaaccgccgaaaaaaggcaaaaagaaaagcagcaaacagaaaaccctggattttctgaacgataccgtgcgcattaccggcgcgagcccgccggaagcgattcagtaa

SEQ ID NO: 28 - DNA, 804 bp, Artificial Sequence
  Nucleic acid sequence encoding gene of mismatch endonuclease variant Q78R+L125V from PF0012
atggaaatgaccaaagcgattgtgaaagaaaacccgcgcattgaagaaattaaagaactgctggaagtggcggaaagccgcgaaggcctgctgaccatttttgcgcgctgcaccgtgtattatgaaggccgcgcgaaaagcgaactgggcgaaggcgatcgcattattattattaaaccggatggcagctttctgattcatcagaaaaagaaacgcgaaccggtgaactggcgcccgccgggcagcaaagtgaaaatggaaggcaacagcctgattagcattcgccgcaacccgaaagaaaccctgaaagtggatattattgaagcgtatgcggcggtgctgtttatggcggaagattatgaagaactgaccgttaccggcagcgaagcggaaatggcggaactgatttttcagaacccgaacgtgattgaagaaggctttaaaccgatgtttcgcgaaaaaccgattaaacatggcattgtggatgtgctgggcgtggatcgcgaaggcaacattgtggtgctggaactgaaacgccgccgcgcggatctgcatgcggtgagccagctgaaacgctatgtggatgcgctgaaagaagaacatggcaacaaagtgcgcggcattctggtggcgccgagcctgaccgaaggcgcgaaaaaactgctggaaaaactgggcctggaatttcgcaaactggaaccgccgaaaaaaggcaaaaagaaaagcagcaaacagaaaaccctggattttctgaacgataccgtgcgcattaccggcgcgagcccgccggaagcgattcagtaa

SEQ ID NO: 29 - DNA, 804 bp, Artificial Sequence
  Nucleic acid sequence encoding gene of mismatch endonuclease variant Q78R+L125A from PF0012
atggaaatgaccaaagcgattgtgaaagaaaacccgcgcattgaagaaattaaagaactgctggaagtggcggaaagccgcgaaggcctgctgaccatttttgcgcgctgcaccgtgtattatgaaggccgcgcgaaaagcgaactgggcgaaggcgatcgcattattattattaaaccggatggcagctttctgattcatcagaaaaagaaacgcgaaccggtgaactggcgcccgccgggcagcaaagtgaaaatggaaggcaacagcctgattagcattcgccgcaacccgaaagaaaccctgaaagtggatattattgaagcgtatgcggcggtgctgtttatggcggaagattatgaagaactgaccgcgaccggcagcgaagcggaaatggcggaactgatttttcagaacccgaacgtgattgaagaaggctttaaaccgatgtttcgcgaaaaaccgattaaacatggcattgtggatgtgctgggcgtggatcgcgaaggcaacattgtggtgctggaactgaaacgccgccgcgcggatctgcatgcggtgagccagctgaaacgctatgtggatgcgctgaaagaagaacatggcaacaaagtgcgcggcattctggtggcgccgagcctgaccgaaggcgcgaaaaaactgctggaaaaactgggcctggaatttcgcaaactggaaccgccgaaaaaaggcaaaaagaaaagcagcaaacagaaaaccctggattttctgaacgataccgtgcgcattaccggcgcgagcccgccggaagcgattcagtaa

SEQ ID NO: 30 - DNA, 1629 bp, Artificial Sequence
  Nucleic acid sequence encoding gene of mismatch endonuclease variant hetero dimer from variant S47R+N76D+L123A and variant Q78R+L123M
atggaaatgaccaaagcgattgtgaaagaaaacccgcgcattgaagaaattaaagaactgctggaagtggcggaaagccgcgaaggcctgctgaccatttttgcgcgctgcaccgtgtattatgaaggccgcgcgaaacgcgaactgggcgaaggcgatcgcattattattattaaaccggatggcagctttctgattcatcagaaaaagaaacgcgaaccggtggattggcagccgccgggcagcaaagtgaaaatggaaggcaacagcctgattagcattcgccgcaacccgaaagaaaccctgaaagtggatattattgaagcgtatgcggcggtgctgtttatggcggaagattatgaagaagcgaccctgaccggcagcgaagcggaaatggcggaactgatttttcagaacccgaacgtgattgaagaaggctttaaaccgatgtttcgcgaaaaaccgattaaacatggcattgtggatgtgctgggcgtggatcgcgaaggcaacattgtggtgctggaactgaaacgccgccgcgcggatctgcatgcggtgagccagctgaaacgctatgtggatgcgctgaaagaagaacatggcaacaaagtgcgcggcattctggtggcgccgagcctgaccgaaggcgcgaaaaaactgctggaaaaactgggcctggaatttcgcaaactggaaccgccgaaaaaaggcaaaaagaaaagcagcaaacagaaaaccctggattttctgaacgataccgtgcgcattaccggcgcgagcccgccggaagcgattcagctggaagttctgttccaggggcccatggaaatgaccaaagcgattgtgaaagaaaacccgcgcattgaagaaattaaagaactgctggaagtggcggaaagccgcgaaggcctgctgaccatttttgcgcgctgcaccgtgtattatgaaggccgcgcgaaaagcgaactgggcgaaggcgatcgcattattattattaaaccggatggcagctttctgattcatcagaaaaagaaacgcgaaccggtgaactggcgcccgccgggcagcaaagtgaaaatggaaggcaacagcctgattagcattcgccgcaacccgaaagaaaccctgaaagtggatattattgaagcgtatgcggcggtgctgtttatggcggaagattatgaagaaatgaccctgaccggcagcgaagcggaaatggcggaactgatttttcagaacccgaacgtgattgaagaaggctttaaaccgatgtttcgcgaaaaaccgattaaacatggcattgtggatgtgctgggcgtggatcgcgaaggcaacattgtggtgctggaactgaaacgccgccgcgcggatctgcatgcggtgagccagctgaaacgctatgtggatgcgctgaaagaagaacatggcaacaaagtgcgcggcattctggtggcgccgagcctgaccgaaggcgcgaaaaaactgctggaaaaactgggcctggaatttcgcaaactggaaccgccgaaaaaaggcaaaaagaaaagcagcaaacagaaaaccctggattttctgaacgataccgtgcgcattaccggcgcgagcccgccggaagcgattcagtaa

SEQ ID NO: 31 - DNA, 23 bp, Artificial Sequence
  Synthetic oligo nucleotide "NucS-Template-T"
aatatccgttaggcattgaagca

SEQ ID NO: 32 - DNA, 23 bp, Artificial Sequence
  Synthetic oligo nucleotide "NucS-Template-G"
aatatccggtaggcattgaagca

SEQ ID NO: 33 - DNA, 15 bp, Artificial Sequence
  Synthetic oligo nucleotide "NucS-Probe-T". 5'-end is labeled with FAM and 3'-end is labeled with Eclipse.
atgcctatcggatat

SEQ ID NO: 34 - DNA, 15 bp, Artificial Sequence
  Synthetic oligo nucleotide "NucS-Probe-G". 5'-end is labeled with FAM and 3'-end is labeled with Eclipse.
atgcctagcggatat

SEQ ID NO: 35 - protein, 8 aa, Artificial Sequence
  Amino acid sequence of Linker
LEVLFQGP

SEQ ID NO: 36 - DNA, 24 bp, Artificial Sequence
  Nucleic acid sequence encoding Linker
ctggaagttctgttccaggggccc